European Patent Specification EP 3 523 647 B1, published June 26, 2024. Title: IDENTIFICATION AND MONITORING OF CLEAVED IMMUNOGLOBULINS BY MOLECULAR MASS. Applicant: Mayo Foundation for Medical Education and Research. The sequence listing filed with the application follows.

SEQUENCE LISTING (3 sequences)

SEQ ID NO: 1 - protein, 22 aa, Homo sapiens
PKSCDKTHTCPPCPAPELLGGP

SEQ ID NO: 2 - protein, 12 aa, Homo sapiens
THTCPPCPAPEL

SEQ ID NO: 3 - protein, 227 aa, Homo sapiens
THTCPPCPAPELLGGPSVFLFPPKPKDTLMISRTPEVTCVVVDVSHEDPEVKFNWYVDGVEVHNAKTKPREEQYNSTYRVVSVLTVLHQDWLNGKEYKCKVSNKALPAPIEKTISKAKGQPREPQVYTLPPSRDELTKNQVSLTCLVKGFYPSDIAVEWESNGQPENNYKTTPPVLDSDGSFFLYSKLTVDKSRWQQGNVFSCSVMHEALHNHYTQKSLSLSPGKGK